European Patent Application EP 4 628 094 A2, published October 8, 2025. Title: BAFF-R ANTIBODIES AND USES THEREOF. Applicant: City of Hope. Application IB PCT/US2017/036181, filed June 6, 2017. The sequence listing filed with the application follows.

SEQUENCE LISTING (32 sequences)

SEQ ID NO: 1 - protein, 10 aa, Mus musculus
ESVDNYGISF

SEQ ID NO: 2 - skipped

SEQ ID NO: 3 - protein, 9 aa, Mus musculus
QQSKEVPWT

SEQ ID NO: 4 - protein, 8 aa, Mus musculus
GDSITSGY

SEQ ID NO: 5 - protein, 7 aa, Mus musculus
ISYSGST

SEQ ID NO: 6 - protein, 12 aa, Mus musculus
ASPNYPFYAMDY

SEQ ID NO: 7 - protein, 6 aa, Mus musculus
QDISNY

SEQ ID NO: 8 - skipped

SEQ ID NO: 9 - protein, 7 aa, Mus musculus
FSELPWT

SEQ ID NO: 10 - protein, 10 aa, Mus musculus
GFSLSTSGMG

SEQ ID NO: 11 - protein, 7 aa, Mus musculus
IWWDDDK

SEQ ID NO: 12 - protein, 10 aa, Mus musculus
ARSFGYGLDY

SEQ ID NO: 13 - DNA, 411 bp, synthetic construct
  misc_feature 1..411: note = synthetic construct
  source 1..411: mol_type = other DNA
atgtacaggatgcaactcctgtcttgcattgcactaagtcttgcacttgtcacgaattcagacattgtgctgacccaatctccagcttctttggctgtgtctctagggcagagggccaccatctcctgcagagccagcgaaagtgttgataattatggcattagttttatgaactggttccaacagaaaccaggacagccacccaaactcctcatctatgctgcatccaaccaaggatccggggtccctgccaggtttagtggcagtgggtctgggacagacttcagcctcaacatccatcctatggaggaggatgatactgcaatgtatttctgtcagcaaagtaaggaggttccgtggacgttcggtggaggcaccaagctggaaatcaaaaccatggaaatcaaacgt

SEQ ID NO: 14 - protein, 137 aa, synthetic construct
  REGION 1..137: note = synthetic construct
MYRMQLLSCIALSLALVTNSDIVLTQSPASLAVSLGQRATISCRASESVDNYGISFMNWFQQKPGQPPKLLIYAASNQGSGVPARFSGSGSGTDFSLNIHPMEEDDTAMYFCQQSKEVPWTFGGGTKLEIKTMEIKR

SEQ ID NO: 15 - DNA, 420 bp, synthetic construct
  misc_feature 1..420: note = synthetic construct
  source 1..420: mol_type = other DNA
atgtacaggatgcaactcctgtcttgcattgcactaagtcttgcacttgtcacgaattcggaggtgcagctgcaggagtctggacctagcctcgtgaaaccttctcagactctgtccctcacctgttctgtcactggcgactccatcaccagtggttactggaactggatccggaaattcccagggaataaacttgagtacatggggtacataagctacagtggtagcacttactacaatccatctctcaaaagtcgaatctccatcactcgagacacatccaagaaccagtactacctgcagttaaattctgtgacacctgaggacacagccacatattactgtgcaagccccaattaccccttctatgctatggactactggggtcaaggaacctcagtcaccgtctcctcagatatc

SEQ ID NO: 16 - protein, 140 aa, synthetic construct
  REGION 1..140: note = synthetic construct
MYRMQLLSCIALSLALVTNSEVQLQESGPSLVKPSQTLSLTCSVTGDSITSGYWNWIRKFPGNKLEYMGYISYSGSTYYNPSLKSRISITRDTSKNQYYLQLNSVTPEDTATYYCASPNYPFYAMDYWGQGTSVTVSSDI

SEQ ID NO: 17 - DNA, 403 bp, synthetic construct
  misc_feature 1..403: note = synthetic construct
  source 1..403: mol_type = other DNA
atggagaccgacaccctgctgctctgggtgctgctgctctgggtgcccggctccaccggagagatcgtgctgacccagagccctgccaccctgtctctgagccctggcgagagagctaccctgtcctgcagagcctccgagtccgtggacaactacggcatctccttcctgaactggttccagcagaagcccggccaggcccccagactgctgatctacgccgcctctaatcgggccaccggcatccctgccagattctccggatctggctccggcaccgactttaccctgaccatctccagcctggaacccgaggacttcgccgtgtactactgccagcagtccaaagaggtgccctggacctttggcggaggcaccaaggtggaaatcaagcggaccgtgg

SEQ ID NO: 18 - protein, 134 aa, synthetic construct
  REGION 1..134: note = synthetic construct
METDTLLLWVLLLWVPGSTGEIVLTQSPATLSLSPGERATLSCRASESVDNYGISFLNWFQQKPGQAPRLLIYAASNRATGIPARFSGSGSGTDFTLTISSLEPEDFAVYYCQQSKEVPWTFGGGTKVEIKRTV

SEQ ID NO: 19 - DNA, 403 bp, synthetic construct
  misc_feature 1..403: note = synthetic construct
  source 1..403: mol_type = other DNA
atggagaccgacaccctgctgctctgggtgctgctgctctgggtgcccggctccaccggagacatcgtgctgacccagagccctgccaccctgtctctgagccctggcgagagagctaccctgtcctgcagagcctccgagtccgtggacaactacggcatctccttcatgaactggttccagcagaagcccggccaggcccccagactgctgatctacgccgcctctaatcgggccaccggcatccctgccagattctccggatctggctccggcaccgactttaccctgaccatctccagcctggaacccgaggacttcgccgtgtactactgccagcagtccaaagaggtgccctggacctttggcggaggcaccaaggtggaaatcaagcggaccgtgg

SEQ ID NO: 20 - protein, 134 aa, synthetic construct
  REGION 1..134: note = synthetic construct
METDTLLLWVLLLWVPGSTGDIVLTQSPATLSLSPGERATLSCRASESVDNYGISFMNWFQQKPGQAPRLLIYAASNRATGIPARFSGSGSGTDFTLTISSLEPEDFAVYYCQQSKEVPWTFGGGTKVEIKRTV

SEQ ID NO: 21 - DNA, 403 bp, synthetic construct
  misc_feature 1..403: note = synthetic construct
  source 1..403: mol_type = other DNA
atggagaccgacaccctgctgctctgggtgctgctgctctgggtgcccggctccaccggagacatcgtgatgacccagagcccctccagcctgtctgcctctgtgggcgacagagtgaccatcacctgtcgggcctccgagtccgtggacaactacggcatctccttcatgaactggttccagcagaagcccggcaaggcccccaagctgctgatctacgccgcctctaatctgggctctggcgtgccctctagattctccggatctggctccggcaccgactttaccctgaccatctccagcctgcagcccgaggacttcgccacctactactgccagcagtccaaagaggtgccctggacctttggccagggcaccaaggtggaaatcaagcggaccgtgg

SEQ ID NO: 22 - protein, 134 aa, synthetic construct
  REGION 1..134: note = synthetic construct
METDTLLLWVLLLWVPGSTGDIVMTQSPSSLSASVGDRVTITCRASESVDNYGISFMNWFQQKPGKAPKLLIYAASNLGSGVPSRFSGSGSGTDFTLTISSLQPEDFATYYCQQSKEVPWTFGQGTKVEIKRTV

SEQ ID NO: 23 - DNA, 426 bp, synthetic construct
  misc_feature 1..426: note = synthetic construct
  source 1..426: mol_type = other DNA
atggaccccaagggcagcctgagctggagaatcctgctgttcctgagcctggccttcgagctgagctacggccaggtgcagctgcaggaatctggccctggcctcgtgaagccttcccagaccctgtccctgacctgcaccgtgtccggcgactctatcacctccggctactggaactggatccggcagcatcctggcaagggcctggagtatatcggctacatctcctactccggctccacctactacaaccccagcctgaagtccagagtgaccatctcccgggacacctccaagaaccagttctccctgaagctgtcctccgtgaccgctgctgataccgccgtgtactactgcgcctcccccaactaccccttctacgccatggactactggggccagggcaccctcgtgaccgtgtcctct

SEQ ID NO: 24 - protein, 142 aa, synthetic construct
  REGION 1..142: note = synthetic construct
MDPKGSLSWRILLFLSLAFELSYGQVQLQESGPGLVKPSQTLSLTCTVSGDSITSGYWNWIRQHPGKGLEYIGYISYSGSTYYNPSLKSRVTISRDTSKNQFSLKLSSVTAADTAVYYCASPNYPFYAMDYWGQGTLVTVSS

SEQ ID NO: 25 - DNA, 426 bp, synthetic construct
  misc_feature 1..426: note = synthetic construct
  source 1..426: mol_type = other DNA
atggaccccaagggcagcctgagctggagaatcctgctgttcctgagcctggccttcgagctgagctacggcgaagtgcagctgcaggaatctggccctggcctcgtgaagccttcccagaccctgtccctgacctgcaccgtgtccggcgactctatcacctccggctactggaactggatccggcagcatcctggcaagggcctggagtatatcggctacatctcctactccggctccacctactacaaccccagcctgaagtccagagtgaccatctcccgggacacctccaagaaccagtactccctgaagctgtcctccgtgaccgctgctgataccgccgtgtactactgcgcctcccccaactaccccttctacgccatggactactggggccagggcaccctcgtgaccgtgtcctct

SEQ ID NO: 26 - protein, 142 aa, synthetic construct
  REGION 1..142: note = synthetic construct
MDPKGSLSWRILLFLSLAFELSYGEVQLQESGPGLVKPSQTLSLTCTVSGDSITSGYWNWIRQHPGKGLEYIGYISYSGSTYYNPSLKSRVTISRDTSKNQYSLKLSSVTAADTAVYYCASPNYPFYAMDYWGQGTLVTVSS

SEQ ID NO: 27 - DNA, 426 bp, synthetic construct
  misc_feature 1..426: note = synthetic construct
  source 1..426: mol_type = other DNA
atggaccccaagggcagcctgagctggagaatcctgctgttcctgagcctggccttcgagctgagctacggcgaagtgcagctgcaggaatctggccctggcctcgtgaagccttccgagaccctgtccctgacctgctccgtgtccggcgactctatcacctccggctactggaactggatccggcagcctcctggcaagggcctggagtatatcggctacatctcctactccggctccacctactacaaccccagcctgaagtccagagtgaccatctcccgggacacctccaagaaccagtactccctgcggctgtcctccgtgaccgctgctgataccgccctgtactactgcgcctcccccaactaccccttctacgccatggactactggggccagggcacaagagtgaccgtgtcctct

SEQ ID NO: 28 - protein, 142 aa, synthetic construct
  REGION 1..142: note = synthetic construct
MDPKGSLSWRILLFLSLAFELSYGEVQLQESGPGLVKPSETLSLTCSVSGDSITSGYWNWIRQPPGKGLEYIGYISYSGSTYYNPSLKSRVTISRDTSKNQYSLRLSSVTAADTALYYCASPNYPFYAMDYWGQGTRVTVSS

SEQ ID NO: 29 - DNA, 387 bp, synthetic construct
  misc_feature 1..387: note = synthetic construct
  source 1..387: mol_type = other DNA
atgtacaggatgcaactcctgtcttgcattgcactaagtcttgcacttgtcacgaattcagatatccagatgacacagactacatcctccctgtctgcctctctgggagacagagtcaccatcagttgcagtgcaagtcaggacattagcaattatttaaactggtatcagcagaaaccagatggaactgttaaactcctgatctattacacatcaagtttacactcaggagtcccatcaaggttcagtggcagtgggtctgggacagattattctctcaccatcagcagcctggaacctgaagatattgccacttactattgtcatcagtttagtgagcttccgtggacgttcggtggaggcaccaagctggaaataaaacgtacg

SEQ ID NO: 30 - protein, 129 aa, synthetic construct
  REGION 1..129: note = synthetic construct
MYRMQLLSCIALSLALVTNSDIQMTQTTSSLSASLGDRVTISCSASQDISNYLNWYQQKPDGTVKLLIYYTSSLHSGVPSRFSGSGSGTDYSLTISSLEPEDIATYYCHQFSELPWTFGGGTKLEIKRT

SEQ ID NO: 31 - DNA, 420 bp, synthetic construct
  misc_feature 1..420: note = synthetic construct
  source 1..420: mol_type = other DNA
atgtacaggatgcaactcctgtcttgcattgcactaagtcttgcacttgtcacgaattcgcaggttactctgaaagagtctggccctgggatattgaagccctcacagaccctcagtctgacttgttctttctctgggttttcactgagcacttctggtatgggtgtaggctggattcgtcagccttcagggaagggtctggagtggctggcacacatttggtgggatgatgataaatactataactcatccctgaagagtcacctcacaatctccaaggatacctccagaaaccaggtattcctcaagatcaccagtgtggacactgcagatactgccacttactactgtgctcgaagctttggttacggtcttgactactggggccaaggcaccactctcacagtctcctcagctagc

SEQ ID NO: 32 - protein, 140 aa, synthetic construct
  REGION 1..140: note = synthetic construct
MYRMQLLSCIALSLALVTNSQVTLKESGPGILKPSQTLSLTCSFSGFSLSTSGMGVGWIRQPSGKGLEWLAHIWWDDDKYYNSSLKSHLTISKDTSRNQVFLKITSVDTADTATYYCARSFGYGLDYWGQGTTLTVSSAS